European Patent Application EP 4 772 533 A1, published July 8, 2026. Title: 重组人源化III型三螺旋胶原蛋白及其制备方法和应用. Applicant: 科兴生物制药股份有限公司. The sequence listing filed with the application follows.

SEQUENCE LISTING (25 sequences)

SEQ ID NO: 1 - protein, 1466 aa, synthetic construct
MMSFVQKGSWLLLALLHPTIILAQQEAVEGGCSHLGQSYADRDVWKPEPCQICVCDSGSVLCDDIICDDQELDCPNPEIPFGECCAVCPQPPTAPTRPPNGQGPQGPKGDPGPPGIPGRNGDPGIPGQPGSPGSPGPPGICESCPTGPQNYSPQYDSYDVKSGVAVGGLAGYPGPAGPPGPPGPPGTSGHPGSPGSPGYQGPPGEPGQAGPSGPPGPPGAIGPSGPAGKDGESGRPGRPGERGLPGPPGIKGPAGIPGFPGMKGHRGFDGRNGEKGETGAPGLKGENGLPGENGAPGPMGPRGAPGERGRPGLPGAAGARGNDGARGSDGQPGPPGPPGTAGFPGSPGAKGEVGPAGSPGSNGAPGQRGEPGPQGHAGAQGPPGPPGINGSPGGKGEMGPAGIPGAPGLMGARGPPGPAGANGAPGLRGGAGEPGKNGAKGEPGPRGERGEAGIPGVPGAKGEDGKDGSPGEPGANGLPGAAGERGAPGFRGPAGPNGIPGEKGPAGERGAPGPAGPRGAAGEPGRDGVPGGPGMRGMPGSPGGPGSDGKPGPPGSQGESGRPGPPGPSGPRGQPGVMGFPGPKGNDGAPGKNGERGGPGGPGPQGPPGKNGETGPQGPPGPTGPGGDKGDTGPPGPQGLQGLPGTGGPPGENGKPGEPGPKGDAGAPGAPGGKGDAGAPGERGPPGLAGAPGLRGGAGPPGPEGGKGAAGPPGPPGAAGTPGLQGMPGERGGLGSPGPKGDKGEPGGPGADGVPGKDGPRGPTGPIGPPGPAGQPGDKGEGGAPGLPGIAGPRGSPGERGETGPPGPAGFPGAPGQNGEPGGKGERGAPGEKGEGGPPGVAGPPGGSGPAGPPGPQGVKGERGSPGGPGAAGFPGARGLPGPPGSNGNPGPPGPSGSPGKDGPPGPAGNTGAPGSPGVSGPKGDAGQPGEKGSPGAQGPPGAPGPLGIAGITGARGLAGPPGMPGPRGSPGPQGVKGESGKPGANGLSGERGPPGPQGLPGLAGTAGEPGRDGNPGSDGLPGRDGSPGGKGDRGENGSPGAPGAPGHPGPPGPVGPAGKSGDRGESGPAGPAGAPGPAGSRGAPGPQGPRGDKGETGERGAAGIKGHRGFPGNPGAPGSPGPAGQQGAIGSPGPAGPRGPVGPSGPPGKDGTSGHPGPIGPPGPRGNRGERGSEGSPGHPGQPGPPGPPGAPGPCCGGVGAAAIAGIGGEKAGGFAPYYGDEPMDFKINTDEIMTSLKSVNGQIESLISPDGSRKNPARNCRDLKFCHPELKSGEYWVDPNQGCKLDAIKVFCNMETGETCISANPLNVPRKHWWTDSSAEKKHVWFGESMDGGFQFSYGNPELPEDVLDVQLAFLRLLSSRASQNITYHCKNSIAYMDQASGNVKKALKLMGSNEGEFKAEGNSKFTYTVLEDGCTKHTGEWSKTVFEYRTRKAVRLPIVDIAPYDIGGPDQEFGVDVGPVCFL

SEQ ID NO: 2 - protein, 84 aa, synthetic construct
GPRGDKGETGERGAAGIKGHRGFPGNPGAPGSPGPAGQQGAIGSPGPAGPRGPVGPSGPPGKDGTSGHPGPIGPPGPRGNRGER

SEQ ID NO: 3 - protein, 514 aa, synthetic construct
GPRGDKGETGERGAAGIKGHRGFPGNPGAPGSPGPAGQQGAIGSPGPAGPRGPVGPSGPPGKDGTSGHPGPIGPPGPRGNRGERGPRGDKGETGERGAAGIKGHRGFPGNPGAPGSPGPAGQQGAIGSPGPAGPRGPVGPSGPPGKDGTSGHPGPIGPPGPRGNRGERGPRGDKGETGERGAAGIKGHRGFPGNPGAPGSPGPAGQQGAIGSPGPAGPRGPVGPSGPPGKDGTSGHPGPIGPPGPRGNRGERGPRGDKGETGERGAAGIKGHRGFPGNPGAPGSPGPAGQQGAIGSPGPAGPRGPVGPSGPPGKDGTSGHPGPIGPPGPRGNRGERGPRGDKGETGERGAAGIKGHRGFPGNPGAPGSPGPAGQQGAIGSPGPAGPRGPVGPSGPPGKDGTSGHPGPIGPPGPRGNRGERGPRGDKGETGERGAAGIKGHRGFPGNPGAPGSPGPAGQQGAIGSPGPAGPRGPVGPSGPPGKDGTSGHPGPIGPPGPRGNRGERGPPGPCCGGG

SEQ ID NO: 4 - DNA, 1542 bp, synthetic construct
  source 1..1542: mol_type = other DNA
ggtccaagaggtgataagggtgaaactggtgaaagaggtgctgctggtattaagggtcatagaggttttccaggtaacccaggtgctccaggttctccaggtccagctggtcaacaaggtgctattggttctccaggtccagctggtccaagaggtccagttggtccatctggtccaccaggtaaggatggtacttctggtcatccaggtccaattggtccaccaggtccaagaggtaacagaggtgaaagaggtccaagaggtgataagggtgaaactggtgaaagaggtgctgctggtattaagggtcatagaggttttccaggtaacccaggtgctccaggttctccaggtccagctggtcaacaaggtgctattggttctccaggtccagctggtccaagaggtccagttggtccatctggtccaccaggtaaggatggtacttctggtcatccaggtccaattggtccaccaggtccaagaggtaacagaggtgaaagaggtccaagaggtgataagggtgaaactggtgaaagaggtgctgctggtattaagggtcatagaggttttccaggtaacccaggtgctccaggttctccaggtccagctggtcaacaaggtgctattggttctccaggtccagctggtccaagaggtccagttggtccatctggtccaccaggtaaggatggtacttctggtcatccaggtccaattggtccaccaggtccaagaggtaacagaggtgaaagaggtccaagaggtgataagggtgaaactggtgaaagaggtgctgctggtattaagggtcatagaggttttccaggtaacccaggtgctccaggttctccaggtccagctggtcaacaaggtgctattggttctccaggtccagctggtccaagaggtccagttggtccatctggtccaccaggtaaggatggtacttctggtcatccaggtccaattggtccaccaggtccaagaggtaacagaggtgaaagaggtccaagaggtgataagggtgaaactggtgaaagaggtgctgctggtattaagggtcatagaggttttccaggtaacccaggtgctccaggttctccaggtccagctggtcaacaaggtgctattggttctccaggtccagctggtccaagaggtccagttggtccatctggtccaccaggtaaggatggtacttctggtcatccaggtccaattggtccaccaggtccaagaggtaacagaggtgaaagaggtccaagaggtgataagggtgaaactggtgaaagaggtgctgctggtattaagggtcatagaggttttccaggtaacccaggtgctccaggttctccaggtccagctggtcaacaaggtgctattggttctccaggtccagctggtccaagaggtccagttggtccatctggtccaccaggtaaggatggtacttctggtcatccaggtccaattggtccaccaggtccaagaggtaacagaggtgaaagaggtccaccaggtccatgttgtggtggtggt

SEQ ID NO: 5 - DNA, 5089 bp, synthetic construct
  source 1..5089: mol_type = other DNA
agatctaacatccaaagacgaaaggttgaatgaaacctttttgccatccgacatccacaggtccattctcacacataagtgccaaacgcaacaggaggggatacactagcagcagaccgttgcaaacgcaggacctccactcctcttctcctcaacacccacttttgccatcgaaaaaccagcccagttattgggcttgattggagctcgctcattccaattccttctattaggctactaacaccatgactttattagcctgtctatcctggcccccctggcgaggttcatgtttgtttatttccgaatgcaacaagctccgcattacacccgaacatcactccagatgagggctttctgagtgtggggtcaaatagtttcatgttccccaaatggcccaaaactgacagtttaaacgctgtcttggaacctaatatgacaaaagcgtgatctcatccaagatgaactaagtttggttcgttgaaatgctaacggccagttggtcaaaaagaaacttccaaaagtcggcataccgtttgtcttgtttggtattgattgacgaatgctcaaaaataatctcattaatgcttagcgcagtctctctatcgcttctgaaccccggtgcacctgtgccgaaacgcaaatggggaaacacccgctttttggatgattatgcattgtctccacattgtatgcttccaagattctggtgggaatactgctgatagcctaacgttcatgatcaaaatttaactgttctaacccctacttgacagcaatatataaacagaaggaagctgccctgtcttaaacctttttttttatcatcattattagcttactttcataattgcgactggttccaattgacaagcttttgattttaacgacttttaacgacaacttgagaagatcaaaaaacaactaattattcgaaacgatgagatttccttcaatttttactgctgttttattcgcagcatcctccgcattagctgctccagtcaacactacaacagaagatgaaacggcacaaattccggctgaagctgtcatcggttactcagatttagaaggggatttcgatgttgctgttttgccattttccaacagcacaaataacgggttattgtttataaatactactattgccagcattgctgctaaagaagaaggggtatctctcgagaagagagaagctgaagctggtccaagaggtgataagggtgaaactggtgaaagaggtgctgctggtattaagggtcatagaggttttccaggtaacccaggtgctccaggttctccaggtccagctggtcaacaaggtgctattggttctccaggtccagctggtccaagaggtccagttggtccatctggtccaccaggtaaggatggtacttctggtcatccaggtccaattggtccaccaggtccaagaggtaacagaggtgaaagaggtccaagaggtgataagggtgaaactggtgaaagaggtgctgctggtattaagggtcatagaggttttccaggtaacccaggtgctccaggttctccaggtccagctggtcaacaaggtgctattggttctccaggtccagctggtccaagaggtccagttggtccatctggtccaccaggtaaggatggtacttctggtcatccaggtccaattggtccaccaggtccaagaggtaacagaggtgaaagaggtccaagaggtgataagggtgaaactggtgaaagaggtgctgctggtattaagggtcatagaggttttccaggtaacccaggtgctccaggttctccaggtccagctggtcaacaaggtgctattggttctccaggtccagctggtccaagaggtccagttggtccatctggtccaccaggtaaggatggtacttctggtcatccaggtccaattggtccaccaggtccaagaggtaacagaggtgaaagaggtccaagaggtgataagggtgaaactggtgaaagaggtgctgctggtattaagggtcatagaggttttccaggtaacccaggtgctccaggttctccaggtccagctggtcaacaaggtgctattggttctccaggtccagctggtccaagaggtccagttggtccatctggtccaccaggtaaggatggtacttctggtcatccaggtccaattggtccaccaggtccaagaggtaacagaggtgaaagaggtccaagaggtgataagggtgaaactggtgaaagaggtgctgctggtattaagggtcatagaggttttccaggtaacccaggtgctccaggttctccaggtccagctggtcaacaaggtgctattggttctccaggtccagctggtccaagaggtccagttggtccatctggtccaccaggtaaggatggtacttctggtcatccaggtccaattggtccaccaggtccaagaggtaacagaggtgaaagaggtccaagaggtgataagggtgaaactggtgaaagaggtgctgctggtattaagggtcatagaggttttccaggtaacccaggtgctccaggttctccaggtccagctggtcaacaaggtgctattggttctccaggtccagctggtccaagaggtccagttggtccatctggtccaccaggtaaggatggtacttctggtcatccaggtccaattggtccaccaggtccaagaggtaacagaggtgaaagaggtccaccaggtccatgttgtggtggtggttaggcggccgccagctttctagaacaaaaactcatctcagaagaggatctgaatagcgccgtcgaccatcatcatcatcatcattgagtttgtagccttagacatgactgttcctcagttcaagttgggcacttacgagaagaccggtcttgctagattctaatcaagaggatgtcagaatgccatttgcctgagagatgcaggcttcatttttgatacttttttatttgtaacctatatagtataggattttttttgtcattttgtttcttctcgtacgagcttgctcctgatcagcctatctcgcagctgatgaatatcttgtggtaggggtttgggaaaatcattcgagtttgatgtttttcttggtatttcccactcctcttcagagtacagaagattaagtgagaccttcgtttgtgcggatcccccacacaccatagcttcaaaatgtttctactccttttttactcttccagattttctcggactccgcgcatcgccgtaccacttcaaaacacccaagcacagcatactaaattttccctctttcttcctctagggtgtcgttaattacccgtactaaaggtttggaaaagaaaaaagagaccgcctcgtttctttttcttcgtcgaaaaaggcaataaaaatttttatcacgtttctttttcttgaaatttttttttttagtttttttctctttcagtgacctccattgatatttaagttaataaacggtcttcaatttctcaagtttcagtttcatttttcttgttctattacaactttttttacttcttgttcattagaaagaaagcatagcaatctaatctaaggggcggtgttgacaattaatcatcggcatagtatatcggcatagtataatacgacaaggtgaggaactaaaccatggccaagttgaccagtgccgttccggtgctcaccgcgcgcgacgtcgccggagcggtcgagttctggaccgaccggctcgggttctcccgggacttcgtggaggacgacttcgccggtgtggtccgggacgacgtgaccctgttcatcagcgcggtccaggaccaggtggtgccggacaacaccctggcctgggtgtgggtgcgcggcctggacgagctgtacgccgagtggtcggaggtcgtgtccacgaacttccgggacgcctccgggccggccatgaccgagatcggcgagcagccgtgggggcgggagttcgccctgcgcgacccggccggcaactgcgtgcacttcgtggccgaggagcaggactgacacgtccgacggcggcccacgggtcccaggcctcggagatccgtcccccttttcctttgtcgatatcatgtaattagttatgtcacgcttacattcacgccctccccccacatccgctctaaccgaaaaggaaggagttagacaacctgaagtctaggtccctatttatttttttatagttatgttagtattaagaacgttatttatatttcaaatttttcttttttttctgtacagacgcgtgtacgcatgtaacattatactgaaaaccttgcttgagaaggttttgggacgctcgaaggctttaatttgcaagctggagaccaacatgtgagcaaaaggccagcaaaaggccaggaaccgtaaaaaggccgcgttgctggcgtttttccataggctccgcccccctgacgagcatcacaaaaatcgacgctcaagtcagaggtggcgaaacccgacaggactataaagataccaggcgtttccccctggaagctccctcgtgcgctctcctgttccgaccctgccgcttaccggatacctgtccgcctttctcccttcgggaagcgtggcgctttctcaatgctcacgctgtaggtatctcagttcggtgtaggtcgttcgctccaagctgggctgtgtgcacgaaccccccgttcagcccgaccgctgcgccttatccggtaactatcgtcttgagtccaacccggtaagacacgacttatcgccactggcagcagccactggtaacaggattagcagagcgaggtatgtaggcggtgctacagagttcttgaagtggtggcctaactacggctacactagaaggacagtatttggtatctgcgctctgctgaagccagttaccttcggaaaaagagttggtagctcttgatccggcaaacaaaccaccgctggtagcggtggtttttttgtttgcaagcagcagattacgcgcagaaaaaaaggatctcaagaagatcctttgatcttttctacggggtctgacgctcagtggaacgaaaactcacgttaagggattttggtcatgagatc

SEQ ID NO: 6 - protein, 10 aa, synthetic construct
GPPGPCCGGG

SEQ ID NO: 7 - protein, 63 aa, synthetic construct
GRPGRPGERGLPGPPGIKGPAGIPGFPGMKGHRGFDGRNGEKGETGAPGLKGENGLPGENGAP

SEQ ID NO: 8 - protein, 39 aa, synthetic construct
GEKGETGAPGLKGENGLPGENGAPGPMGPRGAPGERGRP

SEQ ID NO: 9 - protein, 165 aa, synthetic construct
GLPGENGAPGPMGPRGAPGERGRPGLPGAAGARGNDGARGSDGQPGPPGPPGTAGFPGSPGAKGEVGPAGSPGSNGAPGQRGEPGPQGHAGAQGPPGPPGINGSPGGKGEMGPAGIPGAPGLMGARGPPGPAGANGAPGLRGGAGEPGKNGAKGEPGPRGERGEA

SEQ ID NO: 10 - protein, 186 aa, synthetic construct
GPRGAPGERGRPGLPGAAGARGNDGARGSDGQPGPPGPPGTAGFPGSPGAKGEVGPAGSPGSNGAPGQRGEPGPQGHAGAQGPPGPPGINGSPGGKGEMGPAGIPGAPGLMGARGPPGPAGANGAPGLRGGAGEPGKNGAKGEPGPRGERGEAGIPGVPGAKGEDGKDGSPGEPGANGLPGAAGER

SEQ ID NO: 11 - protein, 60 aa, synthetic construct
GPRGERGEAGIPGVPGAKGEDGKDGSPGEPGANGLPGAAGERGAPGFRGPAGPNGIPGEK

SEQ ID NO: 12 - protein, 30 aa, synthetic construct
GERGAPGFRGPAGPNGIPGEKGPAGERGAP

SEQ ID NO: 13 - protein, 99 aa, synthetic construct
GEKGPAGERGAPGPAGPRGAAGEPGRDGVPGGPGMRGMPGSPGGPGSDGKPGPPGSQGESGRPGPPGPSGPRGQPGVMGFPGPKGNDGAPGKNGERGGP

SEQ ID NO: 14 - protein, 180 aa, synthetic construct
GERGAPGPAGPRGAAGEPGRDGVPGGPGMRGMPGSPGGPGSDGKPGPPGSQGESGRPGPPGPSGPRGQPGVMGFPGPKGNDGAPGKNGERGGPGGPGPQGPPGKNGETGPQGPPGPTGPGGDKGDTGPPGPQGLQGLPGTGGPPGENGKPGEPGPKGDAGAPGAPGGKGDAGAPGERGPP

SEQ ID NO: 15 - protein, 141 aa, synthetic construct
GKNGERGGPGGPGPQGPPGKNGETGPQGPPGPTGPGGDKGDTGPPGPQGLQGLPGTGGPPGENGKPGEPGPKGDAGAPGAPGGKGDAGAPGERGPPGLAGAPGLRGGAGPPGPEGGKGAAGPPGPPGAAGTPGLQGMPGER

SEQ ID NO: 16 - protein, 129 aa, synthetic construct
GAPGERGPPGLAGAPGLRGGAGPPGPEGGKGAAGPPGPPGAAGTPGLQGMPGERGGLGSPGPKGDKGEPGGPGADGVPGKDGPRGPTGPIGPPGPAGQPGDKGEGGAPGLPGIAGPRGSPGERGETGPP

SEQ ID NO: 17 - protein, 105 aa, synthetic construct
GMPGERGGLGSPGPKGDKGEPGGPGADGVPGKDGPRGPTGPIGPPGPAGQPGDKGEGGAPGLPGIAGPRGSPGERGETGPPGPAGFPGAPGQNGEPGGKGERGAP

SEQ ID NO: 18 - protein, 39 aa, synthetic construct
GSPGERGETGPPGPAGFPGAPGQNGEPGGKGERGAPGEK

SEQ ID NO: 19 - protein, 42 aa, synthetic construct
GERGETGPPGPAGFPGAPGQNGEPGGKGERGAPGEKGEGGPP

SEQ ID NO: 20 - protein, 42 aa, synthetic construct
GERGAPGEKGEGGPPGVAGPPGGSGPAGPPGPQGVKGERGSP

SEQ ID NO: 21 - protein, 105 aa, synthetic construct
GAPGEKGEGGPPGVAGPPGGSGPAGPPGPQGVKGERGSPGGPGAAGFPGARGLPGPPGSNGNPGPPGPSGSPGKDGPPGPAGNTGAPGSPGVSGPKGDAGQPGEK

SEQ ID NO: 22 - protein, 135 aa, synthetic construct
GERGSPGGPGAAGFPGARGLPGPPGSNGNPGPPGPSGSPGKDGPPGPAGNTGAPGSPGVSGPKGDAGQPGEKGSPGAQGPPGAPGPLGIAGITGARGLAGPPGMPGPRGSPGPQGVKGESGKPGANGLSGERGPP

SEQ ID NO: 23 - protein, 168 aa, synthetic construct
GQPGEKGSPGAQGPPGAPGPLGIAGITGARGLAGPPGMPGPRGSPGPQGVKGESGKPGANGLSGERGPPGPQGLPGLAGTAGEPGRDGNPGSDGLPGRDGSPGGKGDRGENGSPGAPGAPGHPGPPGPVGPAGKSGDRGESGPAGPAGAPGPAGSRGAPGPQGPRGDK

SEQ ID NO: 24 - protein, 117 aa, synthetic construct
GLSGERGPPGPQGLPGLAGTAGEPGRDGNPGSDGLPGRDGSPGGKGDRGENGSPGAPGAPGHPGPPGPVGPAGKSGDRGESGPAGPAGAPGPAGSRGAPGPQGPRGDKGETGERGAA

SEQ ID NO: 25 - protein, 478 aa, synthetic construct
GSPGERGETGPPGPAGFPGAPGQNGEPGGKGERGAPGEKGSPGERGETGPPGPAGFPGAPGQNGEPGGKGERGAPGEKGSPGERGETGPPGPAGFPGAPGQNGEPGGKGERGAPGEKGSPGERGETGPPGPAGFPGAPGQNGEPGGKGERGAPGEKGSPGERGETGPPGPAGFPGAPGQNGEPGGKGERGAPGEKGSPGERGETGPPGPAGFPGAPGQNGEPGGKGERGAPGEKGSPGERGETGPPGPAGFPGAPGQNGEPGGKGERGAPGEKGSPGERGETGPPGPAGFPGAPGQNGEPGGKGERGAPGEKGSPGERGETGPPGPAGFPGAPGQNGEPGGKGERGAPGEKGSPGERGETGPPGPAGFPGAPGQNGEPGGKGERGAPGEKGSPGERGETGPPGPAGFPGAPGQNGEPGGKGERGAPGEKGSPGERGETGPPGPAGFPGAPGQNGEPGGKGERGAPGEKGPPGPCCGGG